European Patent Specification EP 3 505 535 B1, published October 16, 2024. Title: PD1 Antibody and Pharmaceutical Composition and Use Thereof. Applicant: AKESO BIOPHARMA, INC. The sequence listing filed with the application follows.

SEQUENCE LISTING (14 sequences)

SEQ ID NO: 1 - DNA, 354 bp, Artificial
  Nucleotide sequence of monoclonal antibody 14C12  heavy chain variable region
gaggtcaaactggtggagagcggcggcgggctggtgaagcccggcgggtcactgaaactgagctgcgccgcttccggcttcgcctttagctcctacgacatgtcatgggtgaggcagacccctgagaagcgcctggaatgggtcgctactatcagcggaggcgggcgatacacctactatcctgactctgtcaaagggagattcacaattagtcgggataacgccagaaatactctgtatctgcagatgtctagtctgcggtccgaggatacagctctgtactattgtgcaaaccggtacggcgaagcatggtttgcctattggggacagggcaccctggtgacagtctctgcc

SEQ ID NO: 2 - protein, 118 aa, Artificial
  The amino acid sequence of monoclonal antibody 14C12 heavy chain variable region
EVKLVESGGGLVKPGGSLKLSCAASGFAFSSYDMSWVRQTPEKRLEWVATISGGGRYTYYPDSVKGRFTISRDNARNTLYLQMSSLRSEDTALYYCANRYGEAWFAYWGQGTLVTVSA

SEQ ID NO: 3 - DNA, 318 bp, Artificial
  Nucleotide sequence of monoclonal antibody 14C12 light chain variable region
gacattaagatgacacagtccccttcctcaatgtacgctagcctgggcgagcgagtgaccttcacatgcaaagcatcccaggacatcaacacatacctgtcttggtttcagcagaagccaggcaaaagccccaagaccctgatctaccgggccaatagactggtggacggggtccccagcagattctccggatctggcagtgggcaggattactccctgaccatcagctccctggagtatgaagacatgggcatctactattgcctgcagtatgatgagttccctctgacctttggagcaggcacaaaactggaactg

SEQ ID NO: 4 - protein, 106 aa, Artificial
  The amino acid sequence of monoclonal antibody 14C12 light chain variable region
DIKMTQSPSSMYASLGERVTFTCKASQDINTYLSWFQQKPGKSPKTLIYRANRLVDGVPSRFSGSGSGQDYSLTISSLEYEDMGIYYCLQYDEFPLTFGAGTKLEL

SEQ ID NO: 5 - DNA, 354 bp, Artificial
  Nucleotide sequence of monoclonal antibody 14C12H1L1  heavy chain variable region
gaagtgcagctggtcgagtctgggggagggctggtgcagcccggcgggtcactgcgactgagctgcgcagcttccggattcgcctttagctcctacgacatgtcctgggtgcgacaggcaccaggaaagggactggattgggtcgctactatctcaggaggcgggagatacacctactatcctgacagcgtcaagggccggttcacaatctctagagataacagtaagaacaatctgtatctgcagatgaacagcctgagggctgaggacaccgcactgtactattgtgccaaccgctacggggaagcatggtttgcctattgggggcagggaaccctggtgacagtctctagt

SEQ ID NO: 6 - protein, 118 aa, Artificial
  The amino acid sequence of monoclonal antibody 14C12H1L1 heavy chain variable region
EVQLVESGGGLVQPGGSLRLSCAASGFAFSSYDMSWVRQAPGKGLDWVATISGGGRYTYYPDSVKGRFTISRDNSKNNLYLQMNSLRAEDTALYYCANRYGEAWFAYWGQGTLVTVSS

SEQ ID NO: 7 - DNA, 321 bp, Artificial
  Nucleotide sequence of monoclonal antibody 14C12H1L1 light chain variable region
gacattcagatgactcagagcccctcctccatgtccgcctctgtgggcgacagggtcaccttcacatgccgcgctagtcaggatatcaacacctacctgagctggtttcagcagaagccagggaaaagccccaagacactgatctaccgggctaatagactggtgtctggagtcccaagtcggttcagtggctcagggagcggacaggactacactctgaccatcagctccctgcagcctgaggacatggcaacctactattgcctgcagtatgatgagttcccactgacctttggcgccgggacaaaactggagctgaag

SEQ ID NO: 8 - protein, 107 aa, Artificial
  The amino acid sequence of monoclonal antibody 14C12H1L1 light chain variable region
DIQMTQSPSSMSASVGDRVTFTCRASQDINTYLSWFQQKPGKSPKTLIYRANRLVSGVPSRFSGSGSGQDYTLTISSLQPEDMATYYCLQYDEFPLTFGAGTKLELK

SEQ ID NO: 9 - protein, 8 aa, Artificial
  HCDR
GFAFSSYD

SEQ ID NO: 10 - protein, 8 aa, Artificial
  HCDR
ISGGGRYT

SEQ ID NO: 11 - protein, 11 aa, Artificial
  HCDR
ANRYGEAWFAY

SEQ ID NO: 12 - protein, 6 aa, LCDR
QDINTY

SEQ ID NO: 13 - protein, 3 aa, Artificial
  LCDR
RAN

SEQ ID NO: 14 - protein, 9 aa, Artificial
  LCDR
LQYDEFPLT